European Patent Application EP 4 591 942 A2, published July 30, 2025. Title: INTERLEUKIN 33 (IL-33) INHIBITION FOR TREATMENT OF CANCER, FIBROSIS AND INFLAMMATION. Applicant: The General Hospital Corporation. Application IB PCT/US2021/040725, filed July 7, 2021. The sequence listing filed with the application follows.

SEQUENCE LISTING (21 sequences)

SEQ ID NO: 1 - DNA, 20 bp, synthetic construct
  misc_feature 1..20: note = Smad6 forward primer
  source 1..20: mol_type = other DNA
gcaacccctaccacttcagc

SEQ ID NO: 2 - DNA, 21 bp, synthetic construct
  misc_feature 1..21: note = Smad6 reverse primer
  source 1..21: mol_type = other DNA
gtggcttgtactggtcaggag

SEQ ID NO: 3 - DNA, 22 bp, synthetic construct
  misc_feature 1..22: note = Gapdh forward primer
  source 1..22: mol_type = other DNA
aatgtgtccgtcgtggatctga

SEQ ID NO: 4 - DNA, 22 bp, synthetic construct
  misc_feature 1..22: note = Gapdh reverse primer
  source 1..22: mol_type = other DNA
gatgcctgcttcaccaccttct

SEQ ID NO: 5 - DNA, 25 bp, synthetic construct
  misc_feature 1..25: note = Smad6 promoter forward primer
  source 1..25: mol_type = other DNA
ggactgactctaaagtgctatgcgc

SEQ ID NO: 6 - DNA, 25 bp, synthetic construct
  misc_feature 1..25: note = Smad6 promoter reverse primer
  source 1..25: mol_type = other DNA
acagtgcccgcgactcactctcaag

SEQ ID NO: 7 - DNA, 20 bp, synthetic construct
  misc_feature 1..20: note = Smad6 no peak forward primer
  source 1..20: mol_type = other DNA
gttcagatgatgtggcagaa

SEQ ID NO: 8 - DNA, 21 bp, synthetic construct
  misc_feature 1..21: note = Smad6 no peak reverse primer
  source 1..21: mol_type = other DNA
ctttctaagccctgggaccct

SEQ ID NO: 9 - DNA, 20 bp, synthetic construct
  misc_feature 1..20: note = Smad6 peak forward primer
  source 1..20: mol_type = other DNA
cttggcaatcctcagagaag

SEQ ID NO: 10 - DNA, 21 bp, synthetic construct
  misc_feature 1..21: note = Smad6 peak reverse primer
  source 1..21: mol_type = other DNA
atgagtggattacatagtcag

SEQ ID NO: 11 - DNA, 18 bp, synthetic construct
  misc_feature 1..18: note = IL-33 forward primer
  source 1..18: mol_type = other DNA
gagagatcaaatgaggcc

SEQ ID NO: 12 - DNA, 18 bp, synthetic construct
  misc_feature 1..18: note = IL-33 forward mutant primer
  source 1..18: mol_type = other DNA
ggtcgctaccattaccag

SEQ ID NO: 13 - DNA, 18 bp, synthetic construct
  misc_feature 1..18: note = IL-33 reverse primer
  source 1..18: mol_type = other DNA
gctggagaccagacttgt

SEQ ID NO: 14 - DNA, 22 bp, synthetic construct
  misc_feature 1..22: note = ST2 forward wild-type primer
  source 1..22: mol_type = other DNA
gaagagggcttcactctgtatc

SEQ ID NO: 15 - DNA, 22 bp, synthetic construct
  misc_feature 1..22: note = ST2 reverse wild-type primer
  source 1..22: mol_type = other DNA
ggaggaggaggagttgttaaag

SEQ ID NO: 16 - DNA, 22 bp, synthetic construct
  misc_feature 1..22: note = ST2 forward mutant primer
  source 1..22: mol_type = other DNA
gatctcctgtcatctcaccttg

SEQ ID NO: 17 - DNA, 20 bp, synthetic construct
  misc_feature 1..20: note = ST2 reverse mutant primer
  source 1..20: mol_type = other DNA
gccaacgctatgtcctgata

SEQ ID NO: 18 - DNA, 24 bp, synthetic construct
  misc_feature 1..24: note = K14-IL33 forward primer
  source 1..24: mol_type = other DNA
ggagggggcaaagttttcagggtg

SEQ ID NO: 19 - DNA, 20 bp, synthetic construct
  misc_feature 1..20: note = K14-IL33 reverse primer
  source 1..20: mol_type = other DNA
tttgcaaggcgggaccaggg

SEQ ID NO: 20 - DNA, 25 bp, synthetic construct
  misc_feature 1..25: note = Il33 promoter forward primer
  source 1..25: mol_type = other DNA
gaaactcatgcagactgttgaccaa

SEQ ID NO: 21 - DNA, 23 bp, synthetic construct
  misc_feature 1..23: note = Il33 promoter reverse primer
  source 1..23: mol_type = other DNA
gtgcacgattcttagaaaatgtt